European Patent Specification EP 3 931 349 B1, published December 11, 2024. Title: APOE GENOTYPING IN CANCER PROGNOSTICS AND TREATMENT. Applicant: The Rockefeller University Tavazoie, Sohail Ostendorf, Benjamin N Tavazoie, Masoud Gonsalves, Foster. The sequence listing filed with the application follows.

SEQUENCE LISTING (16 sequences)

SEQ ID NO: 1 - DNA, 951 bp, Homo sapiens
atgaaggttctgtgggctgcgttgctggtcacattcctggcaggatgccaggccaaggtggagcaagcggtggagacagagccggagcccgagctgcgccagcagaccgagtggcagagcggccagcgctgggaactggcactgggtcgcttttgggattacctgcgctgggtgcagacactgtctgagcaggtgcaggaggagctgctcagctcccaggtcacccaggaactgagggcgctgatggacgagaccatgaaggagttgaaggcctacaaatcggaactggaggaacaactgaccccggtggcggaggagacgcgggcacggctgtccaaggagctgcaggcggcgcaggcccggctgggcgcggacatggaggacgtgtgcggccgcctggtgcagtaccgcggcgaggtgcaggccatgctcggccagagcaccgaggagctgcgggtgcgcctcgcctcccacctgcgcaagctgcgtaagcggctcctccgcgatgccgatgacctgcagaagtgcctggcagtgtaccaggccggggcccgcgagggcgccgagcgcggcctcagcgccatccgcgagcgcctggggcccctggtggaacagggccgcgtgcgggccgccactgtgggctccctggccggccagccgctacaggagcgggcccaggcctggggcgagcggctgcgcgcgcggatggaggagatgggcagccggacccgcgaccgcctggacgaggtgaaggagcaggtggcggaggtgcgcgccaagctggaggagcaggcccagcagatacgcctgcaggccgaggccttccaggcccgcctcaagagctggttcgagcccctggtggaagacatgcagcgccagtgggccgggctggtggagaaggtgcaggctgccgtgggcaccagcgccgcccctgtgcccagcgacaatcac

SEQ ID NO: 2 - DNA, 951 bp, Homo sapiens
atgaaggttctgtgggctgcgttgctggtcacattcctggcaggatgccaggccaaggtggagcaagcggtggagacagagccggagcccgagctgcgccagcagaccgagtggcagagcggccagcgctgggaactggcactgggtcgcttttgggattacctgcgctgggtgcagacactgtctgagcaggtgcaggaggagctgctcagctcccaggtcacccaggaactgagggcgctgatggacgagaccatgaaggagttgaaggcctacaaatcggaactggaggaacaactgaccccggtggcggaggagacgcgggcacggctgtccaaggagctgcaggcggcgcaggcccggctgggcgcggacatggaggacgtgtgcggccgcctggtgcagtaccgcggcgaggtgcaggccatgctcggccagagcaccgaggagctgcgggtgcgcctcgcctcccacctgcgcaagctgcgtaagcggctcctccgcgatgccgatgacctgcagaagcgcctggcagtgtaccaggccggggcccgcgagggcgccgagcgcggcctcagcgccatccgcgagcgcctggggcccctggtggaacagggccgcgtgcgggccgccactgtgggctccctggccggccagccgctacaggagcgggcccaggcctggggcgagcggctgcgcgcgcggatggaggagatgggcagccggacccgcgaccgcctggacgaggtgaaggagcaggtggcggaggtgcgcgccaagctggaggagcaggcccagcagatacgcctgcaggccgaggccttccaggcccgcctcaagagctggttcgagcccctggtggaagacatgcagcgccagtgggccgggctggtggagaaggtgcaggctgccgtgggcaccagcgccgcccctgtgcccagcgacaatcac

SEQ ID NO: 3 - DNA, 951 bp, Homo sapiens
atgaaggttctgtgggctgcgttgctggtcacattcctggcaggatgccaggccaaggtggagcaagcggtggagacagagccggagcccgagctgcgccagcagaccgagtggcagagcggccagcgctgggaactggcactgggtcgcttttgggattacctgcgctgggtgcagacactgtctgagcaggtgcaggaggagctgctcagctcccaggtcacccaggaactgagggcgctgatggacgagaccatgaaggagttgaaggcctacaaatcggaactggaggaacaactgaccccggtggcggaggagacgcgggcacggctgtccaaggagctgcaggcggcgcaggcccggctgggcgcggacatggaggacgtgcgcggccgcctggtgcagtaccgcggcgaggtgcaggccatgctcggccagagcaccgaggagctgcgggtgcgcctcgcctcccacctgcgcaagctgcgtaagcggctcctccgcgatgccgatgacctgcagaagcgcctggcagtgtaccaggccggggcccgcgagggcgccgagcgcggcctcagcgccatccgcgagcgcctggggcccctggtggaacagggccgcgtgcgggccgccactgtgggctccctggccggccagccgctacaggagcgggcccaggcctggggcgagcggctgcgcgcgcggatggaggagatgggcagccggacccgcgaccgcctggacgaggtgaaggagcaggtggcggaggtgcgcgccaagctggaggagcaggcccagcagatacgcctgcaggccgaggccttccaggcccgcctcaagagctggttcgagcccctggtggaagacatgcagcgccagtgggccgggctggtggagaaggtgcaggctgccgtgggcaccagcgccgcccctgtgcccagcgacaatcac

SEQ ID NO: 4 - DNA, 23 bp, Artificial
  Synthetic
gcggtctggcagtaaaaactatc

SEQ ID NO: 5 - DNA, 23 bp, Artificial
  Synthetic
gtgaaacagcattgctgtcactt

SEQ ID NO: 6 - DNA, 18 bp, Artificial
  Synthetic
cacgtgggctccagcatt

SEQ ID NO: 7 - DNA, 22 bp, Artificial
  Synthetic
tcaccagtcatttctgcctttg

SEQ ID NO: 8 - DNA, 22 bp, Artificial
  Synthetic
tgagtatttttgtggcaactgc

SEQ ID NO: 9 - DNA, 18 bp, Artificial
  Synthetic
ctctgctgggaaagcggc

SEQ ID NO: 10 - DNA, 20 bp, Artificial
  Synthetic
caagcactctgcgaactgag

SEQ ID NO: 11 - DNA, 21 bp, Artificial
  Synthetic
aagtttttgaaggcaagatgc

SEQ ID NO: 12 - DNA, 22 bp, Artificial
  Synthetic
taccggctcaactaggaaccat

SEQ ID NO: 13 - DNA, 22 bp, Artificial
  Synthetic
tttaatcgtcctccatccctgc

SEQ ID NO: 14 - DNA, 22 bp, Artificial
  Synthetic
gttccatctcagtcccagtctc

SEQ ID NO: 15 - DNA, 26 bp, Artificial
  Synthetic
acagaattcgccccggcctggtacac

SEQ ID NO: 16 - DNA, 25 bp, Artificial
  Synthetic
taagcttggcacggctgtccaagga